European Patent Specification EP 3 498 724 B1, published June 21, 2023. Title: OLIGONUCLEOTIDE CONJUGATE. Applicant: KYOWA HAKKO KIRIN CO., LTD. The sequence listing filed with the application follows.

SEQUENCE LISTING (9 sequences)

SEQ ID NO: 1 - DNA, 16 bp, Artificial Sequence
  CD45-ASO
  misc_feature (1)..(4): LNA
  misc_feature (2)..(16): 5'-phosphonothioate
  misc_feature (13)..(16): LNA
ccaaatgccaagagtt

SEQ ID NO: 2 - DNA, 13 bp, Artificial Sequence
  ApoB-ASO
  misc_feature (1)..(2): LNA
  misc_feature (2)..(2): LNAmC
  misc_feature (2)..(13): 5'-phosphonothioate
  misc_feature (11)..(13): LNA
  misc_feature (12)..(12): LNAmC
gnattggtattna

SEQ ID NO: 3 - DNA, 16 bp, Artificial Sequence
  B2M-ASO
  misc_feature (1)..(4): LNA
  misc_feature (2)..(16): 5'-phosphonothioate
  misc_feature (3)..(3): LNAmC
  misc_feature (13)..(16): LNA
ttntaagcagagtatg

SEQ ID NO: 4 - RNA, 21 nt, Artificial Sequence
  B2M-ssRNA
  modified_base (1)..(1): 2'-deoxy-2'-fluoroadenosine
  modified_base (2)..(2): gm
  modified_base (3)..(3): 2'-deoxy-2'-fluoroguanosine
  modified_base (4)..(4): 2'-O-methyladenosine
  modified_base (5)..(5): 2'-deoxy-2'-fluorocytidine
  modified_base (6)..(6): um
  modified_base (7)..(7): 2'-deoxy-2'-fluoroguanosine
  modified_base (8)..(8): gm
  modified_base (9)..(9): 2'-deoxy-2'-fluorouridine
  modified_base (10)..(10): cm
  modified_base (11)..(12): 2'-deoxy-2'-fluorouridine
  modified_base (13)..(13): um
  modified_base (14)..(14): 2'-deoxy-2'-fluorocytidine
  modified_base (15)..(15): um
  modified_base (16)..(16): 2'-deoxy-2'-fluoroadenosine
  modified_base (17)..(17): um
  modified_base (18)..(18): 2'-deoxy-2'-fluorocytidine
  modified_base (19)..(19): um
  modified_base (20)..(20): 2'-deoxy-2'-fluorocytidine
  misc_feature (20)..(21): 5'-phosphonothioate
  modified_base (21)..(21): um
aggacuggucuuucuaucucu

SEQ ID NO: 5 - RNA, 23 nt, Artificial Sequence
  B2M-as-RNA
  modified_base (1)..(1): 2'-deoxy-2'-fluoroadenosine
  modified_base (2)..(2): gm
  misc_feature (2)..(3): 5'-phosphonothioate
  modified_base (3)..(3): 2'-deoxy-2'-fluoroadenosine
  modified_base (4)..(4): gm
  modified_base (5)..(5): 2'-deoxy-2'-fluoroadenosine
  modified_base (6)..(6): um
  modified_base (7)..(7): 2'-deoxy-2'-fluoroadenosine
  modified_base (8)..(8): gm
  modified_base (9)..(9): 2'-deoxy-2'-fluoroadenosine
  modified_base (10)..(11): 2'-O-methyladenosine
  modified_base (12)..(12): 2'-deoxy-2'-fluoroguanosine
  modified_base (13)..(13): 2'-O-methyladenosine
  modified_base (14)..(14): 2'-deoxy-2'-fluorocytidine
  modified_base (15)..(15): cm
  modified_base (16)..(16): 2'-deoxy-2'-fluoroadenosine
  modified_base (17)..(17): gm
  modified_base (18)..(18): 2'-deoxy-2'-fluorouridine
  modified_base (19)..(19): cm
  modified_base (20)..(20): 2'-deoxy-2'-fluorocytidine
  modified_base (21)..(21): um
  modified_base (22)..(22): 2'-deoxy-2'-fluorouridine
  misc_feature (22)..(23): 5'-phosphonothioate
  modified_base (23)..(23): gm
agagauagaaagaccaguccuug

SEQ ID NO: 6 - RNA, 21 nt, Artificial Sequence
  GAPDH-ssRNA
  modified_base (1)..(1): 2'-deoxy-2'-fluorocytidine
  modified_base (2)..(2): cm
  modified_base (3)..(3): 2'-deoxy-2'-fluorouridine
  modified_base (4)..(4): um
  modified_base (5)..(5): 2'-deoxy-2'-fluorocytidine
  modified_base (6)..(6): 2'-O-methyladenosine
  modified_base (7)..(7): 2'-deoxy-2'-fluorouridine
  modified_base (8)..(8): um
  modified_base (9)..(9): 2'-deoxy-2'-fluoroguanosine
  modified_base (10)..(10): 2'-deoxy-2'-fluoroadenosine
  modified_base (11)..(11): 2'-deoxy-2'-fluorocytidine
  modified_base (12)..(12): cm
  modified_base (13)..(13): 2'-deoxy-2'-fluorouridine
  modified_base (14)..(14): cm
  modified_base (15)..(16): 2'-O-methyladenosine
  modified_base (17)..(17): 2'-deoxy-2'-fluorocytidine
  modified_base (18)..(18): um
  modified_base (19)..(19): 2'-deoxy-2'-fluoroadenosine
  modified_base (20)..(20): cm
  modified_base (21)..(21): 2'-deoxy-2'-fluoroadenosine
ccuucauugaccucaacuaca

SEQ ID NO: 7 - RNA, 21 nt, Artificial Sequence
  GAPDH-as-RNA
  modified_base (1)..(1): um
  modified_base (2)..(2): 2'-deoxy-2'-fluoroadenosine
  modified_base (3)..(3): gm
  modified_base (4)..(4): 2'-deoxy-2'-fluorouridine
  modified_base (5)..(5): um
  modified_base (6)..(6): 2'-deoxy-2'-fluoroguanosine
  modified_base (7)..(7): 2'-deoxy-2'-fluoroadenosine
  modified_base (8)..(8): 2'-deoxy-2'-fluoroguanosine
  modified_base (9)..(9): gm
  modified_base (10)..(10): 2'-deoxy-2'-fluorouridine
  modified_base (11)..(11): cm
  modified_base (12)..(13): 2'-O-methyladenosine
  modified_base (14)..(14): 2'-deoxy-2'-fluorouridine
  modified_base (15)..(15): gm
  modified_base (16)..(16): 2'-deoxy-2'-fluoroadenosine
  modified_base (17)..(17): 2'-O-methyladenosine
  modified_base (18)..(18): 2'-deoxy-2'-fluoroguanosine
  modified_base (19)..(19): gm
  modified_base (20)..(20): 2'-deoxy-2'-fluoroguanosine
  modified_base (21)..(21): gm
  misc_feature (21)..(21): 5'-phosphonothioate
uaguugaggucaaugaagggg

SEQ ID NO: 8 - RNA, 21 nt, Artificial Sequence
  HPRT-1ssRNA
  modified_base (1)..(1): 2'-deoxy-2'-fluorouridine
  modified_base (2)..(2): cm
  modified_base (3)..(3): 2'-deoxy-2'-fluorocytidine
  modified_base (4)..(4): um
  modified_base (5)..(5): 2'-deoxy-2'-fluoroadenosine
  modified_base (6)..(6): um
  modified_base (7)..(7): 2'-deoxy-2'-fluoroguanosine
  modified_base (8)..(8): 2'-O-methyladenosine
  modified_base (9)..(9): 2'-deoxy-2'-fluorocytidine
  modified_base (10)..(10): um
  modified_base (11)..(11): 2'-deoxy-2'-fluoroguanosine
  modified_base (12)..(12): um
  modified_base (13)..(13): 2'-deoxy-2'-fluoroadenosine
  modified_base (14)..(14): gm
  modified_base (15)..(15): 2'-deoxy-2'-fluoroadenosine
  modified_base (16)..(16): um
  modified_base (17)..(17): 2'-deoxy-2'-fluorouridine
  modified_base (18)..(18): um
  modified_base (19)..(19): 2'-deoxy-2'-fluorouridine
  modified_base (20)..(20): 2'-O-methyladenosine
  modified_base (21)..(21): 2'-deoxy-2'-fluorouridine
uccuaugacuguagauuuuau

SEQ ID NO: 9 - RNA, 23 nt, Artificial Sequence
  HPRT-1-as-RNA
  modified_base (1)..(1): 2'-O-methyladenosine
  modified_base (1)..(1): 5'-phosphoryl
  modified_base (2)..(2): 2'-deoxy-2'-fluorouridine
  modified_base (3)..(3): 2'-O-methyladenosine
  modified_base (4)..(4): 2'-deoxy-2'-fluoroadenosine
  modified_base (5)..(5): 2'-O-methyladenosine
  modified_base (6)..(6): 2'-deoxy-2'-fluoroadenosine
  modified_base (7)..(7): um
  modified_base (8)..(8): 2'-deoxy-2'-fluorocytidine
  modified_base (9)..(9): um
  modified_base (10)..(10): 2'-deoxy-2'-fluoroadenosine
  modified_base (11)..(11): cm
  modified_base (12)..(12): 2'-deoxy-2'-fluoroadenosine
  modified_base (13)..(13): gm
  modified_base (14)..(14): 2'-deoxy-2'-fluorouridine
  modified_base (15)..(15): cm
  modified_base (16)..(16): 2'-deoxy-2'-fluoroadenosine
  modified_base (17)..(17): um
  modified_base (18)..(18): 2'-deoxy-2'-fluoroadenosine
  modified_base (19)..(19): gm
  modified_base (20)..(20): 2'-deoxy-2'-fluoroguanosine
  modified_base (21)..(21): 2'-O-methyladenosine
  modified_base (22)..(22): 2'-deoxy-2'-fluoroadenosine
  misc_feature (22)..(23): 5'-phosphonothioate
  modified_base (23)..(23): um
auaaaaucuacagucauaggaau